European Patent Application EP 4 606 901 A1, published August 27, 2025. Title: 产生人源化抗体的动物模型及其构建方法. Applicant: 江苏集萃药康生物科技股份有限公司. Application WO. The sequence listing filed with the application follows.

SEQUENCE LISTING (75 sequences)

SEQ ID NO: 1 - DNA, 20 bp, synthetic construct
  misc_feature 1..20: note = primer
  source 1..20: mol_type = other DNA
actccgaggcacatgcttag

SEQ ID NO: 2 - DNA, 26 bp, synthetic construct
  misc_feature 1..26: note = primer
  source 1..26: mol_type = other DNA
tcctacatcgaagctgaaagcacgag

SEQ ID NO: 3 - DNA, 28 bp, synthetic construct
  misc_feature 1..28: note = primer
  source 1..28: mol_type = other DNA
tacacatttcttctcaagcactggctat

SEQ ID NO: 4 - DNA, 29 bp, synthetic construct
  misc_feature 1..29: note = primer
  source 1..29: mol_type = other DNA
cttcgtctcttctgttatttggcgactcc

SEQ ID NO: 5 - DNA, 24 bp, synthetic construct
  misc_feature 1..24: note = primer
  source 1..24: mol_type = other DNA
ctgtgtagacctcaaagtcagcca

SEQ ID NO: 6 - DNA, 25 bp, synthetic construct
  misc_feature 1..25: note = primer
  source 1..25: mol_type = other DNA
acctccaacagttatcctgcgttaa

SEQ ID NO: 7 - DNA, 22 bp, synthetic construct
  misc_feature 1..22: note = primer
  source 1..22: mol_type = other DNA
aggtaagaatggcctctccagg

SEQ ID NO: 8 - DNA, 21 bp, synthetic construct
  misc_feature 1..21: note = primer
  source 1..21: mol_type = other DNA
aagaaccagccggatctgcaa

SEQ ID NO: 9 - DNA, 20 bp, synthetic construct
  misc_feature 1..20: note = primer
  source 1..20: mol_type = other DNA
cctaccggtggatgtggaat

SEQ ID NO: 10 - DNA, 23 bp, synthetic construct
  misc_feature 1..23: note = primer
  source 1..23: mol_type = other DNA
gtgcggaacattcctcacaaatc

SEQ ID NO: 11 - DNA, 26 bp, synthetic construct
  misc_feature 1..26: note = primer
  source 1..26: mol_type = other DNA
attcaataaactctttccccttgacc

SEQ ID NO: 12 - DNA, 27 bp, synthetic construct
  misc_feature 1..27: note = primer
  source 1..27: mol_type = other DNA
tgctatttgaacataaactaggccaac

SEQ ID NO: 13 - DNA, 25 bp, synthetic construct
  misc_feature 1..25: note = primer
  source 1..25: mol_type = other DNA
tagttgccagccatctgttgtttgc

SEQ ID NO: 14 - DNA, 32 bp, synthetic construct
  misc_feature 1..32: note = primer
  source 1..32: mol_type = other DNA
tgatgtgagcaccttggctaccattgcttatg

SEQ ID NO: 15 - DNA, 30 bp, synthetic construct
  misc_feature 1..30: note = primer
  source 1..30: mol_type = other DNA
cataaacgcacaaacatacagatatatgct

SEQ ID NO: 16 - DNA, 24 bp, synthetic construct
  misc_feature 1..24: note = primer
  source 1..24: mol_type = other DNA
taaatggcatgatgtacgcacctt

SEQ ID NO: 17 - DNA, 30 bp, synthetic construct
  misc_feature 1..30: note = primer
  source 1..30: mol_type = other DNA
cactcacacataaaagttgacactggcact

SEQ ID NO: 18 - DNA, 32 bp, synthetic construct
  misc_feature 1..32: note = primer
  source 1..32: mol_type = other DNA
tcttaaatccctgatcttgctcatctgtgtcg

SEQ ID NO: 19 - DNA, 34 bp, synthetic construct
  misc_feature 1..34: note = primer
  source 1..34: mol_type = other DNA
atgctgatgataaaaccacacagaaaataccttg

SEQ ID NO: 20 - DNA, 36 bp, synthetic construct
  misc_feature 1..36: note = primer
  source 1..36: mol_type = other DNA
ttaataggaggcttcctcacaatgaaacttttagaa

SEQ ID NO: 21 - DNA, 22 bp, synthetic construct
  misc_feature 1..22: note = primer
  source 1..22: mol_type = other DNA
gtccccgtcctcaccattcagt

SEQ ID NO: 22 - DNA, 27 bp, synthetic construct
  misc_feature 1..27: note = primer
  source 1..27: mol_type = other DNA
tgacctgggtttaacctgtcctggaac

SEQ ID NO: 23 - DNA, 30 bp, synthetic construct
  misc_feature 1..30: note = primer
  source 1..30: mol_type = other DNA
tgacactgtggttataataactccccgaac

SEQ ID NO: 24 - DNA, 26 bp, synthetic construct
  misc_feature 1..26: note = primer
  source 1..26: mol_type = other DNA
gcaagggaaggctcccaaacagacga

SEQ ID NO: 25 - DNA, 28 bp, synthetic construct
  misc_feature 1..28: note = primer
  source 1..28: mol_type = other DNA
aaggatgtgatcaagtccctgccgcaaa

SEQ ID NO: 26 - DNA, 29 bp, synthetic construct
  misc_feature 1..29: note = primer
  source 1..29: mol_type = other DNA
actgaagaacatctcctagcagcaacacc

SEQ ID NO: 27 - DNA, 39 bp, synthetic construct
  misc_feature 1..39: note = primer
  source 1..39: mol_type = other DNA
ttcatgtttgaaggataatttcaccagctatactgttcg

SEQ ID NO: 28 - DNA, 36 bp, synthetic construct
  misc_feature 1..36: note = primer
  source 1..36: mol_type = other DNA
attgacttttaaaatgcagtgtagatatgtcagaga

SEQ ID NO: 29 - DNA, 26 bp, synthetic construct
  misc_feature 1..26: note = primer
  source 1..26: mol_type = other DNA
tcccgagtagctggaactatagatgc

SEQ ID NO: 30 - DNA, 21 bp, synthetic construct
  misc_feature 1..21: note = primer
  source 1..21: mol_type = other DNA
atcatgccaagcacagccgta

SEQ ID NO: 31 - DNA, 23 bp, synthetic construct
  misc_feature 1..23: note = primer
  source 1..23: mol_type = other DNA
ccaggagaaattccccacgtcca

SEQ ID NO: 32 - DNA, 38 bp, synthetic construct
  misc_feature 1..38: note = primer
  source 1..38: mol_type = other DNA
acctataaaacattaacttagaacaggggttcaattca

SEQ ID NO: 33 - DNA, 25 bp, synthetic construct
  misc_feature 1..25: note = primer
  source 1..25: mol_type = other DNA
ggctgattttcacagttatggaccc

SEQ ID NO: 34 - DNA, 29 bp, synthetic construct
  misc_feature 1..29: note = primer
  source 1..29: mol_type = other DNA
tccctactgttaagccacaaatcatcgta

SEQ ID NO: 35 - DNA, 23 bp, synthetic construct
  misc_feature 1..23: note = primer
  source 1..23: mol_type = other DNA
ttcctgaccttcttcccgtgtcc

SEQ ID NO: 36 - DNA, 28 bp, synthetic construct
  misc_feature 1..28: note = primer
  source 1..28: mol_type = other DNA
ctgtgctcagcaaagaggagaacttact

SEQ ID NO: 37 - DNA, 26 bp, synthetic construct
  misc_feature 1..26: note = primer
  source 1..26: mol_type = other DNA
aagacttcagagcacagactaagagc

SEQ ID NO: 38 - DNA, 27 bp, synthetic construct
  misc_feature 1..27: note = primer
  source 1..27: mol_type = other DNA
tggtctcccatgattctgttcccaggt

SEQ ID NO: 39 - DNA, 27 bp, synthetic construct
  misc_feature 1..27: note = primer
  source 1..27: mol_type = other DNA
caggtgctgaacagataccagtttcac

SEQ ID NO: 40 - DNA, 27 bp, synthetic construct
  misc_feature 1..27: note = primer
  source 1..27: mol_type = other DNA
tcacggagtgtctcacagtaacagtgc

SEQ ID NO: 41 - DNA, 40 bp, synthetic construct
  misc_feature 1..40: note = primer
  source 1..40: mol_type = other DNA
tcgagtacatttatattttgaagtcctataatcaagcctt

SEQ ID NO: 42 - DNA, 30 bp, synthetic construct
  misc_feature 1..30: note = primer
  source 1..30: mol_type = other DNA
agtttcttattcaagccttataattgctca

SEQ ID NO: 43 - DNA, 26 bp, synthetic construct
  misc_feature 1..26: note = primer
  source 1..26: mol_type = other DNA
cacatcttcttttcagatcagctcgt

SEQ ID NO: 44 - DNA, 24 bp, synthetic construct
  misc_feature 1..24: note = primer
  source 1..24: mol_type = other DNA
ttttatctggggtctgccgtctcc

SEQ ID NO: 45 - DNA, 26 bp, synthetic construct
  misc_feature 1..26: note = primer
  source 1..26: mol_type = other DNA
gctcacactgacttctccttaccgta

SEQ ID NO: 46 - DNA, 30 bp, synthetic construct
  misc_feature 1..30: note = primer
  source 1..30: mol_type = other DNA
gcacactaggcatgtccaattcttacctgg

SEQ ID NO: 47 - DNA, 32 bp, synthetic construct
  misc_feature 1..32: note = primer
  source 1..32: mol_type = other DNA
gctggatgtcttagaaagagctcaaggtcctt

SEQ ID NO: 48 - DNA, 35 bp, synthetic construct
  misc_feature 1..35: note = primer
  source 1..35: mol_type = other DNA
aaggaaactgtatacataatgaaggactagatagg

SEQ ID NO: 49 - DNA, 29 bp, synthetic construct
  misc_feature 1..29: note = primer
  source 1..29: mol_type = other DNA
aatattagccaatggactatgagagtgac

SEQ ID NO: 50 - DNA, 30 bp, synthetic construct
  misc_feature 1..30: note = primer
  source 1..30: mol_type = other DNA
taaaagatccaaatgaaaagccaaggcaac

SEQ ID NO: 51 - DNA, 31 bp, synthetic construct
  misc_feature 1..31: note = primer
  source 1..31: mol_type = other DNA
tcactgagatctttacttcctttatcacgtt

SEQ ID NO: 52 - DNA, 35 bp, synthetic construct
  misc_feature 1..35: note = primer
  source 1..35: mol_type = other DNA
attatgttttatagtatatgtaagtgcaaactggg

SEQ ID NO: 53 - DNA, 30 bp, synthetic construct
  misc_feature 1..30: note = primer
  source 1..30: mol_type = other DNA
gacatgctaaagaaaatttgccaaatagcg

SEQ ID NO: 54 - DNA, 27 bp, synthetic construct
  misc_feature 1..27: note = primer
  source 1..27: mol_type = other DNA
aactacaggacagagataaacggccta

SEQ ID NO: 55 - DNA, 40 bp, synthetic construct
  misc_feature 1..40: note = primer
  source 1..40: mol_type = other DNA
ggagctaaagttgacaaataaaattgtatgtatttaaggt

SEQ ID NO: 56 - DNA, 27 bp, synthetic construct
  misc_feature 1..27: note = primer
  source 1..27: mol_type = other DNA
tctgtacatctttgaggtttgccggtt

SEQ ID NO: 57 - DNA, 33 bp, synthetic construct
  misc_feature 1..33: note = primer
  source 1..33: mol_type = other DNA
gcacatcaacaaaataaatagacagctatccag

SEQ ID NO: 58 - DNA, 28 bp, synthetic construct
  misc_feature 1..28: note = primer
  source 1..28: mol_type = other DNA
agatatcgctggagcatctatatctctg

SEQ ID NO: 59 - DNA, 21 bp, synthetic construct
  misc_feature 1..21: note = primer
  source 1..21: mol_type = other DNA
ctgtgcatccagacccacgag

SEQ ID NO: 60 - DNA, 25 bp, synthetic construct
  misc_feature 1..25: note = primer
  source 1..25: mol_type = other DNA
cccctaatatcctgagtgtcccgtg

SEQ ID NO: 61 - DNA, 32 bp, synthetic construct
  misc_feature 1..32: note = primer
  source 1..32: mol_type = other DNA
atattcctgatgaacatagacctgaaagtcct

SEQ ID NO: 62 - DNA, 34 bp, synthetic construct
  misc_feature 1..34: note = primer
  source 1..34: mol_type = other DNA
gttggataggattttgttcttgattatactctca

SEQ ID NO: 63 - DNA, 29 bp, synthetic construct
  misc_feature 1..29: note = primer
  source 1..29: mol_type = other DNA
ctgtggctactttctcatcttaaggacga

SEQ ID NO: 64 - DNA, 23 bp, synthetic construct
  misc_feature 1..23: note = primer
  source 1..23: mol_type = other DNA
ggtaacaacccatcacacggctt

SEQ ID NO: 65 - DNA, 26 bp, synthetic construct
  misc_feature 1..26: note = primer
  source 1..26: mol_type = other DNA
gcacgtttgtctccagcacctaagtt

SEQ ID NO: 66 - DNA, 20 bp, synthetic construct
  misc_feature 1..20: note = primer
  source 1..20: mol_type = other DNA
tcccctggtgcatgaactct

SEQ ID NO: 67 - DNA, 20 bp, synthetic construct
  misc_feature 1..20: note = primer
  source 1..20: mol_type = other DNA
cattccagggctcaaggcat

SEQ ID NO: 68 - DNA, 25 bp, synthetic construct
  misc_feature 1..25: note = primer
  source 1..25: mol_type = other DNA
gtggcatgtccatctgtagcttgtc

SEQ ID NO: 69 - DNA, 28 bp, synthetic construct
  misc_feature 1..28: note = primer
  source 1..28: mol_type = other DNA
tccactgtgttgtgtgtaggctcatctg

SEQ ID NO: 70 - DNA, 32 bp, synthetic construct
  misc_feature 1..32: note = primer
  source 1..32: mol_type = other DNA
caggtatttctttacaattcaataatggacga

SEQ ID NO: 71 - DNA, 30 bp, synthetic construct
  misc_feature 1..30: note = primer
  source 1..30: mol_type = other DNA
cacagatagattgagaattttccaagcctt

SEQ ID NO: 72 - DNA, 30 bp, synthetic construct
  misc_feature 1..30: note = primer
  source 1..30: mol_type = other DNA
gatgttgtattagtccattctcacggtgct

SEQ ID NO: 73 - DNA, 33 bp, synthetic construct
  misc_feature 1..33: note = primer
  source 1..33: mol_type = other DNA
agccaagaaataaagacaagtttctacaaccac

SEQ ID NO: 74 - DNA, 24 bp, synthetic construct
  misc_feature 1..24: note = primer
  source 1..24: mol_type = other DNA
aacaaaccaggggtcttagtgatg

SEQ ID NO: 75 - DNA, 24 bp, synthetic construct
  misc_feature 1..24: note = primer
  source 1..24: mol_type = other DNA
ggctagatgcctttctcccttgac